European Patent Application EP 4 342 483 A1, published March 27, 2024. Title: An Antiviral Composition Comprising a Nucleolin-Binding Peptide. Applicant: ANYGEN CO., LTD. The sequence listing filed with the application follows.

SEQUENCE LISTING (82 sequences)

SEQ ID NO: 1 - protein, 9 aa, Artificial Sequence
  AGM-330
RHGAMVYLK

SEQ ID NO: 2 - protein, 9 aa, Artificial Sequence
  AGM-331
ADHRHRRSG

SEQ ID NO: 3 - protein, 9 aa, Artificial Sequence
  AGM-332
AVARARRRR

SEQ ID NO: 4 - protein, 9 aa, Artificial Sequence
  AGM-333
RFLKNKKAR

SEQ ID NO: 5 - protein, 9 aa, Artificial Sequence
  AGM-334
RWLKNKKAR

SEQ ID NO: 6 - protein, 9 aa, Artificial Sequence
  AGM-335
FGRLKKPLK

SEQ ID NO: 7 - protein, 9 aa, Artificial Sequence
  AGM-336
KRRRRERAG

SEQ ID NO: 8 - protein, 9 aa, Artificial Sequence
  AGM-337
KRRRKAPTD

SEQ ID NO: 9 - protein, 9 aa, Artificial Sequence
  AGM-330
KHGAMVYLK

SEQ ID NO: 10 - protein, 9 aa, Artificial Sequence
  AGM-330
RRGAMVYLK

SEQ ID NO: 11 - protein, 9 aa, Artificial Sequence
  AGM-330
RHGLMVYLK

SEQ ID NO: 12 - protein, 9 aa, Artificial Sequence
  AGM-330
RHGALVYLK

SEQ ID NO: 13 - protein, 9 aa, Artificial Sequence
  AGM-330
RHGAXVYLK

SEQ ID NO: 14 - protein, 9 aa, Artificial Sequence
  AGM-330
RHGAMAYLK

SEQ ID NO: 15 - protein, 9 aa, Artificial Sequence
  AGM-330
RHGAMVFLK

SEQ ID NO: 16 - protein, 7 aa, Artificial Sequence
  AGM-330
GAMVYLK

SEQ ID NO: 17 - protein, 11 aa, Artificial Sequence
  AGM-330
RHRHGAMVYLK

SEQ ID NO: 18 - protein, 13 aa, Artificial Sequence
  AGM-330
RHRHRHGAMVYLK

SEQ ID NO: 19 - protein, 9 aa, Artificial Sequence
  AGM-330
KLYVMAGHR

SEQ ID NO: 20 - protein, 13 aa, Artificial Sequence
  AGM-330
RHGAMVYLKLKLK

SEQ ID NO: 21 - protein, 11 aa, Artificial Sequence
  TAT
YGRKKRRQRRR

SEQ ID NO: 22 - protein, 13 aa, Artificial Sequence
  TAT(48-60)
GRKKRRQRRRPPQ

SEQ ID NO: 23 - protein, 9 aa, Artificial Sequence
  TAT(49-57)
RKKRRQRRR

SEQ ID NO: 24 - protein, 16 aa, Artificial Sequence
  Penetratin
RQIKIWFQNRRMKWKK

SEQ ID NO: 25 - protein, 8 aa, Artificial Sequence
  R8
RRRRRRRR

SEQ ID NO: 26 - protein, 13 aa, Artificial Sequence
  R9-TAT
GRRRRRRRRRPPQ

SEQ ID NO: 27 - protein, 21 aa, Artificial Sequence
  Pep-1
KETWWETWWTEWSQPKKKRKV

SEQ ID NO: 28 - protein, 11 aa, Artificial Sequence
  Hph-1
YARVRRRGPRR

SEQ ID NO: 29 - protein, 18 aa, Artificial Sequence
  MAP
KLALKLALKALKAALKLA

SEQ ID NO: 30 - protein, 18 aa, Artificial Sequence
  pVEC
LLIILRRRIRKQAHAHSK

SEQ ID NO: 31 - protein, 20 aa, Artificial Sequence
  DS4
VQIFRIMRILRILKLARHST

SEQ ID NO: 32 - protein, 27 aa, Artificial Sequence
  Transportan
GWTLNSAGYLLGKINLKALAALAKKIL

SEQ ID NO: 33 - protein, 20 aa, Artificial Sequence
  gH625
HGLASTLTRWAHYNALIRAF

SEQ ID NO: 34 - protein, 17 aa, Artificial Sequence
  VP22
NAKTRRHERRRKLAIER

SEQ ID NO: 35 - protein, 20 aa, Artificial Sequence
  DS4
VQIFRIMRILRILKLARHST

SEQ ID NO: 36 - protein, 16 aa, Artificial Sequence
  DS4-1
RIMRILRILKLARHST

SEQ ID NO: 37 - protein, 17 aa, Artificial Sequence
  DS4-2
VQIFRIMRILRILKLAR

SEQ ID NO: 38 - protein, 13 aa, Artificial Sequence
  DS4-3
RIMRILRILKLAR

SEQ ID NO: 39 - protein, 17 aa, Artificial Sequence
  KS4
FRLVRLLRFLRILLIIS

SEQ ID NO: 40 - protein, 14 aa, Artificial Sequence
  KS4-1
FRLVRLLRFLRILL

SEQ ID NO: 41 - protein, 10 aa, Artificial Sequence
  KS4-2
RLVRLLRFLR

SEQ ID NO: 42 - protein, 3 aa, Artificial Sequence
  N1
RIL

SEQ ID NO: 43 - protein, 9 aa, Artificial Sequence
  N3
RILRILRIL

SEQ ID NO: 44 - protein, 15 aa, Artificial Sequence
  N5
RILRILRILRILRIL

SEQ ID NO: 45 - protein, 21 aa, Artificial Sequence
  N7
RILRILRILRILRILRILRIL

SEQ ID NO: 46 - protein, 13 aa, Artificial Sequence
  K3
RIFWVIKLARHFI

SEQ ID NO: 47 - protein, 16 aa, Artificial Sequence
  C3
KSLRVLRVLRPLKTIK

SEQ ID NO: 48 - protein, 15 aa, Artificial Sequence
  C4
RLFRVMRLVKLLSRG

SEQ ID NO: 49 - protein, 15 aa, Artificial Sequence
  S2
RSFRLLRVFKLAKSW

SEQ ID NO: 50 - protein, 22 aa, Artificial Sequence
  S4
RVIRLARIGRILRLVKGAKGIR

SEQ ID NO: 51 - protein, 13 aa, Artificial Sequence
  D1
RAGRILRILKLAR

SEQ ID NO: 52 - protein, 13 aa, Artificial Sequence
  D2
RIMRGLRILKLAR

SEQ ID NO: 53 - protein, 13 aa, Artificial Sequence
  D3
RIMRILRLMKLAR

SEQ ID NO: 54 - protein, 13 aa, Artificial Sequence
  D4
RIMRILRILKMFR

SEQ ID NO: 55 - protein, 13 aa, Artificial Sequence
  D5
RIMRILRALKLAR

SEQ ID NO: 56 - protein, 13 aa, Artificial Sequence
  D6
RIMRGMRILKLAR

SEQ ID NO: 57 - protein, 13 aa, Artificial Sequence
  D7
RLFRILRILKLAR

SEQ ID NO: 58 - protein, 13 aa, Artificial Sequence
  D8
RIMRMVRILKLAR

SEQ ID NO: 59 - protein, 13 aa, Artificial Sequence
  D9
RIMRILRLVKLAR

SEQ ID NO: 60 - protein, 13 aa, Artificial Sequence
  D10
RIMRILRILKGVR

SEQ ID NO: 61 - protein, 13 aa, Artificial Sequence
  D11
RNLRILRILKLAR

SEQ ID NO: 62 - protein, 13 aa, Artificial Sequence
  D12
RIMRDIRILKLAR

SEQ ID NO: 63 - protein, 13 aa, Artificial Sequence
  D13
RIMRILRELKLAR

SEQ ID NO: 64 - protein, 13 aa, Artificial Sequence
  D14
RIMRILRILKQLR

SEQ ID NO: 65 - protein, 13 aa, Artificial Sequence
  D15
RIMRILRHMKLAR

SEQ ID NO: 66 - protein, 13 aa, Artificial Sequence
  D16
RIMRSVRILKLAR

SEQ ID NO: 67 - protein, 13 aa, Artificial Sequence
  D17
RTMRILRILKLAR

SEQ ID NO: 68 - protein, 13 aa, Artificial Sequence
  D18
RIMRYARILKLAR

SEQ ID NO: 69 - protein, 13 aa, Artificial Sequence
  D19
RIMRILRQIKLAR

SEQ ID NO: 70 - protein, 13 aa, Artificial Sequence
  D20
RIMRILRILKEVR

SEQ ID NO: 71 - DNA, 20 bp, Artificial Sequence
  primer
ctgccagaagacaatgaacc

SEQ ID NO: 72 - DNA, 20 bp, Artificial Sequence
  primer
ggccattgcttccaatacac

SEQ ID NO: 73 - DNA, 21 bp, Artificial Sequence
  primer
tggatcaagattagagttggc

SEQ ID NO: 74 - DNA, 20 bp, Artificial Sequence
  primer
ccttgtccattcttctgacc

SEQ ID NO: 75 - DNA, 20 bp, Artificial Sequence
  primer
gctatgctcagatcgccagt

SEQ ID NO: 76 - DNA, 22 bp, Artificial Sequence
  primer
tctcgtaagagtccgctagctc

SEQ ID NO: 77 - DNA, 24 bp, Artificial Sequence
  primer
tagaccaaataacgttgaagttga

SEQ ID NO: 78 - DNA, 22 bp, Artificial Sequence
  primer
gattcacaaactgcagattcaa

SEQ ID NO: 79 - DNA, 19 bp, Artificial Sequence
  primer
cacctccagatgccgtttg

SEQ ID NO: 80 - DNA, 20 bp, Artificial Sequence
  primer
atgcgtggttatcatttgcc

SEQ ID NO: 81 - DNA, 20 bp, Artificial Sequence
  primer
cgaaagggaaaaacaaacgc

SEQ ID NO: 82 - DNA, 24 bp, Artificial Sequence
  primer
tcactcactgtcataggtgtcacc